European Patent Application EP 4 368 251 A2, published May 15, 2024. Title: THERAPEUTIC CONJUGATE. Applicant: Porton Biopharma Limited. The sequence listing filed with the application follows.

SEQUENCE LISTING (5 sequences)

SEQ ID NO: 1 - protein, 348 aa, Escherichia coli
MEFFKKTALAALVMGFSGAALALPNITILATGGTIAGGGDSATKSNYTVGKVGVENLVNAVPQLKDIANVKGEQVVNIGSQDMNDNVWLTLAKKINTDCDKTDGFVITHGTDTMEETAYFLDLTVKCDKPVVMVGAMRPSTSMSADGPFNLYNAVVTAADKASANRGVLVVMNDTVLDGRDVTKTNTTDVATFKSVNYGPLGYIHNGKIDYQRTPARKHTSDTPFDVSKLNELPKVGIVYNYANASDLPAKALVDAGYDGIVSAGVGNGNLYKSVFDTLATAAKTGTAVVRSSRVPTGATTQDAEVDDAKYGFVASGTLNPQKARVLLQLALTQTKDPQQIQQIFNQY

SEQ ID NO: 2 - protein, 327 aa, Erwinia chrysanthemi
ADKLPNIVILATGGTIAGSAATGTQTTGYKAGALGVDTLINAVPEVKKLANVKGEQFSNMASENMTGDVVLKLSQRVNELLARDDVDGVVITHGTDTVEESAYFLHLTVKSDKPVVFVAAMRPATAISADGPMNLLEAVRVAGDKQSRGRGVMVVLNDRIGSARYITKTNASTLDTFKANEEGYLGVIIGNRIYYQNRIDKLHTTRSVFDVRGLTSLPKVDILYGYQDDPEYLYDAAIQHGVKGIVYAGMGAGSVSVRGIAGMRKAMEKGVVVIRSTRTGNGIVPPDEELPGLVSDSLNPAHARILLMLALTRTSDPKVIQEYFHTY

SEQ ID NO: 3 - protein, 329 aa, Pseudomonas putida
MIDHSSLPRLSIASLGGTVSMQAQAVGCGVTPTLDCEQQLLQVPQLRQMAQLNVASLCLVPSASLDFATLLDVLAWARCEVERGAQALVVSQGTDSLEESAYFLDLLWPFDAPLVMTGAMRSASQPGNDGPANLLAAAQVALAQGSCGRGVLVVMNDQVHRAARVRKTASMAIAAFESPGCGPLGEVVEGKVVYRHPPARGEVLPVPHRTDQRVALLEACLDADTALLQAVAPLGYEGLVIAGFGAGHVAASWSDVLEQLAPTLPVVVATRTGNGPTARATYGFAGAEIDLQKKGVYMAGHLCPRKCRILLWLLIGTDRRHELHDWLHA

SEQ ID NO: 4 - protein, 325 aa, Pseudomonas fluorescens
MQSANNVMVLYTGGTIGMQASANGLAPASGFEVRMREQFADADLPAWRFREMSPLIDSANMNPAYWQRLRSAVVEAVDAGCDAVLILHGTDTLAYSAAAMSFQLLGLPAPVVFTGSMLPAGVPDSDAWENVSGALTALAEGLEPGVHLYFHGALMAPTRCAKIRSFGRNPFAALQRKDDFARAETLPAALDYRQPKALANVGVLPLIPGFDAAQLDAIISSGIQGLVLECFGSGTGPSDNPQFLASLQRAQDQGVVVVAITQCHEGGVELDVYEAGSRLRGAGVLSGAGMTREAAFGKLHALLGAGLAVEEVRRLVELDLHTNPT

SEQ ID NO: 5 - protein, 330 aa, Wolinella succinogenes
MAKPQVTILATGGTIAGSGESSVKSSYSAGAVTVDKLLAAVPAINDLATIKGEQISSIGSQEMTGKVWLKLAKRVNELLAQKETEAVIITHGTDTMEETAFFLNLTVKSQKPVVLVGAMRSGSSMSADGPMNLYNAVNVAINKASTNKGVVIVMNDEIHAAREATKLNTTAVNAFASPNTGKIGTVYYGKVEYFTQSVRPHTLASEFDISKIEELPRVDILYAHPDDTDVLVNAALQAGAKGIIHAGMGNGNPFPLTQNALEKAAKSGVVVARSSRVGSGSTTQEAEVDDKKLGFVATESLNPQKARVLLMLALTKTSDREAIQKIFSTY